European Patent Specification EP 4 168 581 B1, published September 13, 2023. Title: ADVANCED DUMBBELL PCR FOR ISOMIR DETECTION. Applicant: Hummingbird Diagnostics GmbH. The sequence listing filed with the application follows.

SEQUENCE LISTING (29 sequences)

SEQ ID NO: 1 - DNA, 43 bp, synthetic construct
  misc_feature 1..43: note = 5' adapter
  misc_feature 1..9: note = n is a, c, g, t, u, or is absent
  misc_feature 10..15: note = n is a, c, g, t or u
  misc_feature 16..21: note = Between 1 and 6 nucleotides in positions 16 to 21 can beLNA-enhanced
  misc_feature 38..43: note = Between 1 and 6 nucleotides in positions 38 to 43 can beLNA-enhanced
  misc_RNA 42..43
  source 1..43: mol_type = other DNA
nnnnnnnnnnnnnnncgtggcgtggagtgtgtgctttgccacg

SEQ ID NO: 2 - DNA, 48 bp, synthetic construct
  misc_feature 1..48: note = 3' adapter
  misc_feature 1..8: note = Between 1 and 8 nucleotides in posiitions 1 to 8 can beLNA-enhanced
  misc_feature 1: note = This nucleotide is 5' terminally phosphorylated
  misc_feature 25..32: note = Between 1 and 8 nucleotides in posiitions 25 to 32 can beLNA-enhanced
  misc_feature 33..38: note = n is a, c, g, or t
  misc_feature 39..47: note = n is a, c, g, t, u, or is absent
  misc_feature 48: note = This nucleotide is a 3' inverted deoxynucleotide
  source 1..48: mol_type = other DNA
ctcagtgcagggtccgaggtattcgcactgagnnnnnnnnnnnnnnnt

SEQ ID NO: 3 - DNA, 24 bp, synthetic construct
  misc_feature 1..24: note = RT primer
  source 1..24: mol_type = other DNA
ctcagtgcgaatacctcggaccct

SEQ ID NO: 4 - DNA, 21 bp, synthetic construct
  misc_feature 1..21: note = Forward primer
  source 1..21: mol_type = other DNA
tggagtgtgtgctttgccacg

SEQ ID NO: 5 - DNA, 18 bp, synthetic construct
  misc_feature 1..18: note = Reverse primer
  source 1..18: mol_type = other DNA
gtgcgaatacctcggacc

SEQ ID NO: 6 - DNA, 39 bp, synthetic construct
  misc_feature 1..39: note = Exemplary 5' adapter
  misc_feature 12..17: note = Between 1 and 6 nucleotides in positions 12 to 17 can beLNA-enhanced
  misc_feature 34..39: note = Between 1 and 6 nucleotides in positions 34 to 39 can beLNA-enhanced
  misc_RNA 38..39
  source 1..39: mol_type = other DNA
atctacgggttcgtggcgtggagtgtgtgctttgccacg

SEQ ID NO: 7 - DNA, 40 bp, synthetic construct
  misc_feature 1..40: note = Exemplary 3' adapter
  misc_feature 1: note = This nucleotide is 5' terminally phosphorylated
  misc_feature 1..8: note = Between 1 and 8 nucleotides in posiitions 1 to 8 can beLNA-enhanced
  misc_feature 25..32: note = Between 1 and 8 nucleotides in posiitions 25 to 32 can beLNA-enhanced
  misc_feature 40: note = This nucleotide is a 3' inverted deoxynucleotide
  source 1..40: mol_type = other DNA
ctcagtgcagggtccgaggtattcgcactgagcacaagtt

SEQ ID NO: 8 - RNA, 22 nt, Homo sapiens
  source 1..22: mol_type = other RNA
aacccgtagatccgaacttgtg

SEQ ID NO: 9 - RNA, 21 nt, Homo sapiens
  source 1..21: mol_type = other RNA
acccgtagatccgaacttgtg

SEQ ID NO: 10 - RNA, 23 nt, Homo sapiens
  source 1..23: mol_type = other RNA
aaacccgtagatccgaacttgtg

SEQ ID NO: 11 - RNA, 21 nt, Homo sapiens
  source 1..21: mol_type = other RNA
aacccgtagatccgaacttgt

SEQ ID NO: 12 - RNA, 23 nt, Homo sapiens
  source 1..23: mol_type = other RNA
aacccgtagatccgaacttgtgg

SEQ ID NO: 13 - RNA, 22 nt, Homo sapiens
  source 1..22: mol_type = other RNA
aacgcgtagatccgaacttgtg

SEQ ID NO: 14 - RNA, 22 nt, Homo sapiens
  source 1..22: mol_type = other RNA
aacccgtagatgcgaacttgtg

SEQ ID NO: 15 - RNA, 22 nt, Homo sapiens
  source 1..22: mol_type = other RNA
aacccgtagatccgaactagtg

SEQ ID NO: 16 - DNA, 40 bp, synthetic construct
  misc_feature 1..40: note = 5' adapter DB-mir100-5A for ligation
  misc_feature 19: note = This nucleotide lacks a base
  misc_RNA 39..40
  source 1..40: mol_type = other DNA
atctacgggttcgtggcgntggagtgtgtgctttgccacg

SEQ ID NO: 17 - DNA, 40 bp, synthetic construct
  misc_feature 1..40: note = 5' adapter DB-mir100-5B for ligation
  misc_feature 19: note = This nucleotide lacks a base
  misc_RNA 39..40
  source 1..40: mol_type = other DNA
gatctacgggtcgtggcgntggagtgtgtgctttgccacg

SEQ ID NO: 18 - DNA, 40 bp, synthetic construct
  misc_feature 1..40: note = 5' adapter DB-mir100-5D for ligation
  misc_feature 19: note = This nucleotide lacks a base
  misc_RNA 39..40
  source 1..40: mol_type = other DNA
tctacgggtttcgtggcgntggagtgtgtgctttgccacg

SEQ ID NO: 19 - DNA, 40 bp, synthetic construct
  misc_feature 1..40: note = 5' adapter DB-mir100-5E for ligation
  misc_feature 19: note = This nucleotide lacks a base
  misc_RNA 39..40
  source 1..40: mol_type = other DNA
atctacgcgttcgtggcgntggagtgtgtgctttgccacg

SEQ ID NO: 20 - DNA, 40 bp, synthetic construct; identical to SEQ ID NO: 7
  misc_feature 1..40: note = 3' adapter DB-mir100-3Z for ligation
  misc_feature 1: note = This nucleotide is 5' terminally phosphorylated
  misc_feature 40: note = This nucleotide is a 3' inverted deoxynucleotide
  source 1..40: mol_type = other DNA

SEQ ID NO: 21 - DNA, 40 bp, synthetic construct
  misc_feature 1..40: note = 3' adapter DB-mir100-3X for ligation
  misc_feature 1: note = This nucleotide is 5' terminally phosphorylated
  misc_feature 40: note = This nucleotide is a 3' inverted deoxynucleotide
  source 1..40: mol_type = other DNA
ctcagtgcagggtccgaggtattcgcactgagacaagttt

SEQ ID NO: 22 - DNA, 40 bp, synthetic construct
  misc_feature 1..40: note = 3' adapter DB-mir100-3S for ligation
  misc_feature 1: note = This nucleotide is 5' terminally phosphorylated
  misc_feature 40: note = This nucleotide is a 3' inverted deoxynucleotide
  source 1..40: mol_type = other DNA
ctcagtgcagggtccgaggtattcgcactgagccacaagt

SEQ ID NO: 23 - DNA, 40 bp, synthetic construct
  misc_feature 1..40: note = 3' adapter DB-mir100-3T for ligation
  misc_feature 1: note = This nucleotide is 5' terminally phosphorylated
  misc_feature 40: note = This nucleotide is a 3' inverted deoxynucleotide
  source 1..40: mol_type = other DNA
ctcagtgcagggtccgaggtattcgcactgagcactagtt

SEQ ID NO: 24 - DNA, 20 bp, synthetic construct
  misc_feature 1..20: note = Taqman probe DB-mir100-K
  misc_feature 1: note = Labelled with 5' 6-FAM (fluorescein)
  misc_feature 9..10: note = These two nucleotides are connected by an internal ZEN(TM)quencher, proprietary to Integrated DNA Technologies Inc.
  misc_feature 20: note = Labelled with Iowa black fluorescein quencher
  source 1..20: mol_type = other DNA
acgaacccgtagatccgaac

SEQ ID NO: 25 - DNA, 20 bp, synthetic construct
  misc_feature 1..20: note = Taqman probe DB-mir100-L
  misc_feature 1: note = Labelled with 5' 6-FAM (fluorescein)
  misc_feature 9..10: note = These two nucleotides are connected by an internal ZEN(TM)quencher, proprietary to Integrated DNA Technologies Inc.
  misc_feature 20: note = Labelled with Iowa black fluorescein quencher
  source 1..20: mol_type = other DNA
acgacccgtagatccgaact

SEQ ID NO: 26 - DNA, 20 bp, synthetic construct
  misc_feature 1..20: note = DB-mir100-P
  misc_feature 1: note = Labelled with 5' 6-FAM (fluorescein)
  misc_feature 9..10: note = These two nucleotides are connected by an internal ZEN(TM)quencher, proprietary to Integrated DNA Technologies Inc.
  misc_feature 20: note = Labelled with Iowa black fluorescein quencher
  source 1..20: mol_type = other DNA
acgaaacccgtagatccgaa

SEQ ID NO: 27 - DNA, 20 bp, synthetic construct
  misc_feature 1..20: note = Taqman probe DB-mir100-Q
  misc_feature 1: note = Labelled with 5' 6-FAM (fluorescein)
  misc_feature 9..10: note = These two nucleotides are connected by an internal ZEN(TM)quencher, proprietary to Integrated DNA Technologies Inc.
  misc_feature 20: note = Labelled with Iowa black fluorescein quencher
  source 1..20: mol_type = other DNA
acgaacgcgtagatccgaac

SEQ ID NO: 28 - DNA, 20 bp, synthetic construct
  misc_feature 1..20: note = Taqman probe DB-mir100-R
  misc_feature 1: note = Labelled with 5' 6-FAM (fluorescein)
  misc_feature 9..10: note = These two nucleotides are connected by an internal ZEN(TM)quencher, proprietary to Integrated DNA Technologies Inc.
  misc_feature 20: note = Labelled with Iowa black fluorescein quencher
  source 1..20: mol_type = other DNA
acgaacccgtagatgcgaac

SEQ ID NO: 29 - DNA, 44 bp, synthetic construct
  misc_feature 1..44: note = 5' adapter with idSp
  misc_feature 1..9: note = n is a, c, g, t, u, or is absent
  misc_feature 10..15: note = n is a, c, g, t or u
  misc_feature 16..21: note = Between 1 and 6 nucleotides in positions 16 to 21 can beLNA-enhanced
  misc_feature 23: note = This nucleotide lacks a base
  misc_feature 39..44: note = Between 1 and 6 nucleotides in positions 39 to 44 can beLNA-enhanced
  misc_RNA 43..44
  source 1..44: mol_type = other DNA
nnnnnnnnnnnnnnncgtggcgntggagtgtgtgctttgccacg